European Patent Application EP 4 299 759 A1, published January 3, 2024. Title: Nucleic acid detection method. Applicant: FUNDACION DEL SECTOR PUBLICO ESTATAL CENTRO NACIONAL DE INVESTIGACIONES ONCOLOGICAS CARLOS III (F.S.P. CNIO). The sequence listing filed with the application follows.

SEQUENCE LISTING (10 sequences)

SEQ ID NO: 1 - RNA, 41 nt, Artificial Sequence
  Lba Cas12a guide RNA
uaauuucuacuaaguguagauauagaaaaguccuagguuga

SEQ ID NO: 2 - DNA, 75 bp, SARS coronavirus
  single stranded DNA Lba Cas12a target sequence in SARSCoV2 S gene
cggccgtcgttttacattttttcaacctaggacttttctattaaaatataatttttcaggaaacagctatgaatt

SEQ ID NO: 3 - RNA, 41 nt, Artificial Sequence
  Lba Cas12a guide RNA
uaauuucuacuaaguguagaugaucguuacgcuaacuauga

SEQ ID NO: 4 - DNA, 40 bp, Artificial Sequence
  Amplifier Target Strand
  misc_feature 1..5: /note="phosphorothioate"
  misc_feature 35..39: /note="phosphorothioate"
agccctcatagttagcgtaacgatctgctgttttgtaatc

SEQ ID NO: 5 - DNA, 48 bp, Artificial Sequence
  /note="Amplifier Non target strand" /note="Amplifier Non Target strand"
  misc_feature 1..3: /note="phosphorothioate"
  misc_feature 43..47: /note="phosphorothioate"
gattacaaaacagcagatcgttacgctaactatgagggctuuuuuuuu

SEQ ID NO: 6 - RNA, 64 nt, Artificial Sequence
  Lwa Cas13a guide RNA
gauuuagacuaccccaaaaacgaaggggacuaaaacgcagcaccagcuguccaaccugaagaag

SEQ ID NO: 7 - DNA, 196 bp, Artificial Sequence
  T7 promoter and partial SARS-CoV2 S gene
taatacgactcactataggtaacatcactaggtttcaaactttacttgctttacatagaagttatttgactcctggtgattcttcttcaggttggacagctggtgctgcagcttattatgtgggttatcttcaacctaggacttttctattaaaatataatgaaaatggaaccattacagatgctgtagactgtgc

SEQ ID NO: 8 - DNA, 39 bp, Artificial Sequence
  Amplifier target strand
  misc_feature 1..3: /note="phosphorothioate"
  misc_feature 33..38: /note="phosphorothioate"
cggagtacgcggcatcttgtcagccttggacatgctgat

SEQ ID NO: 9 - DNA, 49 bp, Artificial Sequence
  Amplifier Non target strand
  misc_feature 1..3: /note="phosphorothioate"
  misc_feature 43..47: /note="phosphorothioate"
gattacaaaactttagatcgttacgctaactatgagccgcgtactccgt

SEQ ID NO: 10 - DNA, 49 bp, Artificial Sequence; identical to SEQ ID NO: 9
  Amplifier Target strand